European Patent Application EP 4 299 073 A2, published January 3, 2024. Title: HUMANIZED AND AFFINITY MATURED ANTIBODIES TO FcRH5 AND METHODS OF USE. Applicant: F. Hoffmann-La Roche AG. Application EP, filed June 16, 2016. The sequence listing filed with the application follows.

SEQUENCE LISTING (215 sequences)

SEQ ID NO: 1 - protein, 5 aa, synthetic construct
  REGION 1..5: note = Synthetic construct
RFGVH

SEQ ID NO: 2 - protein, 16 aa, synthetic construct
  REGION 1..16: note = Synthetic construct
  SITE 12: note = MISC_FEATURE - X is A or P
  SITE 15: note = MISC_FEATURE - X is M, G, or V
  SITE 16: note = MISC_FEATURE - X is S, D, or P
VIWRGGSTDYNXAFXX

SEQ ID NO: 3 - protein, 12 aa, synthetic construct
  REGION 1..12: note = Synthetic construct
  SITE 6: note = MISC_FEATURE - X is S or P
HYYGSXDYALDN

SEQ ID NO: 4 - protein, 11 aa, synthetic construct
  REGION 1..11: note = Synthetic construct
  SITE 7: note = MISC_FEATURE - X is S orR
  SITE 9: note = MISC_FEATURE - X is I or L
KASQDVXNXVV

SEQ ID NO: 5 - skipped

SEQ ID NO: 6 - protein, 9 aa, synthetic construct
  REGION 1..9: note = Synthetic construct
  SITE 3: note = MISC_FEATURE - X is H or Q
  SITE 4: note = MISC_FEATURE - X is Y or F
  SITE 5: note = MISC_FEATURE - X is Q or S
  SITE 6: note = MISC_FEATURE - X is S or P
QQXXXXPYT

SEQ ID NO: 7 - protein, 16 aa, synthetic construct
  REGION 1..16: note = Synthetic construct
VIWRGGSTDYNAAFMS

SEQ ID NO: 8 - protein, 16 aa, synthetic construct
  REGION 1..16: note = Synthetic construct
VIWRGGSTDYNAAFVS

SEQ ID NO: 9 - protein, 12 aa, synthetic construct
  REGION 1..12: note = Synthetic construct
HYYGSSDYALDN

SEQ ID NO: 10 - protein, 12 aa, synthetic construct
  REGION 1..12: note = Synthetic construct
HYYGSPDYALDN

SEQ ID NO: 11 - protein, 11 aa, synthetic construct
  REGION 1..11: note = Synthetic construct
KASQDVSNIVV

SEQ ID NO: 12 - protein, 11 aa, synthetic construct
  REGION 1..11: note = Synthetic construct
KASQDVRNLVV

SEQ ID NO: 13 - protein, 11 aa, synthetic construct
  REGION 1..11: note = Synthetic construct
KASQDVRNIVV

SEQ ID NO: 14 - protein, 11 aa, synthetic construct
  REGION 1..11: note = Synthetic construct
KASQDVSNLVV

SEQ ID NO: 15 - protein, 7 aa, synthetic construct
  REGION 1..7: note = Synthetic construct
SASYRYT

SEQ ID NO: 16 - protein, 7 aa, synthetic construct
  REGION 1..7: note = Synthetic construct
SGSYRYS

SEQ ID NO: 17 - protein, 7 aa, synthetic construct
  REGION 1..7: note = Synthetic construct
SGYNRYS

SEQ ID NO: 18 - protein, 7 aa, synthetic construct
  REGION 1..7: note = Synthetic construct
SGYYRYT

SEQ ID NO: 19 - protein, 7 aa, synthetic construct
  REGION 1..7: note = Synthetic construct
SGYYRYS

SEQ ID NO: 20 - protein, 9 aa, synthetic construct
  REGION 1..9: note = Synthetic construct
QQHYSSPYT

SEQ ID NO: 21 - protein, 9 aa, synthetic construct
  REGION 1..9: note = Synthetic construct
QQQYSPPYT

SEQ ID NO: 22 - protein, 9 aa, synthetic construct
  REGION 1..9: note = Synthetic construct
QQQFQPPYT

SEQ ID NO: 23 - protein, 9 aa, synthetic construct
  REGION 1..9: note = Synthetic construct
QQHYSPPYT

SEQ ID NO: 24 - protein, 9 aa, synthetic construct
  REGION 1..9: note = Synthetic construct
QQQYQPPYT

SEQ ID NO: 25 - protein, 9 aa, synthetic construct
  REGION 1..9: note = Synthetic construct
QQHYQPPYT

SEQ ID NO: 26 - protein, 10 aa, synthetic construct
  REGION 1..10: note = Synthetic construct
GIDLSSYAMG

SEQ ID NO: 27 - protein, 16 aa, synthetic construct
  REGION 1..16: note = Synthetic construct
TIGTGGTPYYASWAKG

SEQ ID NO: 28 - protein, 13 aa, synthetic construct
  REGION 1..13: note = Synthetic construct
ARDMYTGSIYYDM

SEQ ID NO: 29 - protein, 13 aa, synthetic construct
  REGION 1..13: note = Synthetic construct
QSSQSVFNNAQLS

SEQ ID NO: 30 - protein, 7 aa, synthetic construct
  REGION 1..7: note = Synthetic construct
DTSNLAS

SEQ ID NO: 31 - protein, 11 aa, synthetic construct
  REGION 1..11: note = Synthetic construct
LGAYTDDADNA

SEQ ID NO: 32 - protein, 10 aa, synthetic construct
  REGION 1..10: note = Synthetic construct
GYTFTHYAMH

SEQ ID NO: 33 - protein, 17 aa, synthetic construct
  REGION 1..17: note = Synthetic construct
MISSSSGNTNFNQKFMD

SEQ ID NO: 34 - protein, 11 aa, synthetic construct
  REGION 1..11: note = Synthetic construct
ARWSYYALFDY

SEQ ID NO: 35 - protein, 10 aa, synthetic construct
  REGION 1..10: note = Synthetic construct
SADSSVDYIH

SEQ ID NO: 36 - protein, 7 aa, synthetic construct
  REGION 1..7: note = Synthetic construct
DTSKLAS

SEQ ID NO: 37 - protein, 9 aa, synthetic construct
  REGION 1..9: note = Synthetic construct
FQGSGYPLT

SEQ ID NO: 38 - protein, 10 aa, synthetic construct
  REGION 1..10: note = Synthetic construct
GYTFTNYVIH

SEQ ID NO: 39 - protein, 17 aa, synthetic construct
  REGION 1..17: note = Synthetic construct
YISPYNDYTKYNEKFEG

SEQ ID NO: 40 - protein, 11 aa, synthetic construct
  REGION 1..11: note = Synthetic construct
ARRDYYGSSDY

SEQ ID NO: 41 - protein, 10 aa, synthetic construct
  REGION 1..10: note = Synthetic construct
SASSSVDYMH

SEQ ID NO: 42 - protein, 7 aa, synthetic construct
  REGION 1..7: note = Synthetic construct
DTSKLAS

SEQ ID NO: 43 - protein, 9 aa, synthetic construct
  REGION 1..9: note = Synthetic construct
QQWSSNPPT

SEQ ID NO: 44 - protein, 30 aa, synthetic construct
  REGION 1..30: note = Synthetic construct
  SITE 1: note = MISC_FEATURE - X is E, S, or F
  SITE 28: note = MISC_FEATURE - X is S or P
  SITE 29: note = MISC_FEATURE - X is L or T
XVQLVESGPGLVKPSETLSLTCTVSGFXXT

SEQ ID NO: 45 - protein, 14 aa, synthetic construct
  REGION 1..14: note = Synthetic construct
  SITE 2: note = MISC_FEATURE - X is V or Y
  SITE 13: note = MISC_FEATURE - X is L or I
WXRQPPGKGLEWXG

SEQ ID NO: 46 - protein, 32 aa, synthetic construct
  REGION 1..32: note = Synthetic construct
RLTISKDNSKNQVSLKLSSVTAADTAVYYCSN

SEQ ID NO: 47 - protein, 11 aa, synthetic construct
  REGION 1..11: note = Synthetic construct
WGQGTLVTVSS

SEQ ID NO: 48 - protein, 23 aa, synthetic construct
  REGION 1..23: note = Synthetic construct
DIQMTQSPSSLSASVGDRVTITC

SEQ ID NO: 49 - protein, 15 aa, synthetic construct
  REGION 1..15: note = Synthetic construct
  SITE 9: note = MISC_FEATURE - X is A or S
WFQQKPGKXPKLLIY

SEQ ID NO: 50 - protein, 32 aa, synthetic construct
  REGION 1..32: note = Synthetic construct
GVPSRFSGSGSGTDFTLTISSLQPEDFATYYC

SEQ ID NO: 51 - protein, 10 aa, synthetic construct
  REGION 1..10: note = Synthetic construct
FGQGTKVEIK

SEQ ID NO: 52 - protein, 30 aa, synthetic construct
  REGION 1..30: note = Synthetic construct
EVQLVESGPGLVKPSETLSLTCTVSGFSLT

SEQ ID NO: 53 - protein, 30 aa, synthetic construct
  REGION 1..30: note = Synthetic construct
EVQLVESGPGLVKPSETLSLTCTVSGFSTT

SEQ ID NO: 54 - protein, 14 aa, synthetic construct
  REGION 1..14: note = Synthetic construct
WVRQPPGKGLEWLG

SEQ ID NO: 55 - protein, 14 aa, synthetic construct
  REGION 1..14: note = Synthetic construct
WVRQPPGKGLEWIG

SEQ ID NO: 56 - protein, 15 aa, synthetic construct
  REGION 1..15: note = Synthetic construct
WFQQKPGKSPKLLIY

SEQ ID NO: 57 - protein, 15 aa, synthetic construct
  REGION 1..15: note = Synthetic construct
WFQQKPGKAPKLLIY

SEQ ID NO: 58 - protein, 25 aa, synthetic construct [sequence omitted]

SEQ ID NO: 59 - protein, 14 aa, synthetic construct
  REGION 1..14: note = Synthetic construct
WVRQAPGKGLEWIG

SEQ ID NO: 60 - protein, 30 aa, synthetic construct
  REGION 1..30: note = Synthetic construct
RFTISKDSSKNTVYLQMNSLRAEDTAVYFC

SEQ ID NO: 61 - protein, 11 aa, synthetic construct
  REGION 1..11: note = Synthetic construct
WGQGTLVTVSS

SEQ ID NO: 62 - protein, 22 aa, synthetic construct
  REGION 1..22: note = Synthetic construct
DAQLTQSPSSLSASVGDRVTIT

SEQ ID NO: 63 - protein, 15 aa, synthetic construct
  REGION 1..15: note = Synthetic construct
WYQQKPGKPPKLLIY

SEQ ID NO: 64 - protein, 32 aa, synthetic construct; identical to SEQ ID NO: 50
  REGION 1..32: note = Synthetic construct

SEQ ID NO: 65 - protein, 10 aa, synthetic construct
  REGION 1..10: note = Synthetic construct
FGQGTKVEIK

SEQ ID NO: 66 - protein, 25 aa, synthetic construct
  REGION 1..25: note = Synthetic construct
QVQLQQSGPELVRPGVSVKISCKGS

SEQ ID NO: 67 - protein, 14 aa, synthetic construct
  REGION 1..14: note = Synthetic construct
WVKQSHTKSLEWIG

SEQ ID NO: 68 - protein, 30 aa, synthetic construct
  REGION 1..30: note = Synthetic construct
KATMTVDKSSTTAYLELARLTFGDSAIYYC

SEQ ID NO: 69 - protein, 11 aa, synthetic construct
  REGION 1..11: note = Synthetic construct
WGQGTTVTVSS

SEQ ID NO: 70 - protein, 23 aa, synthetic construct
  REGION 1..23: note = Synthetic construct
ENVLTQSPAIMSASPGEKVTMTC

SEQ ID NO: 71 - protein, 15 aa, synthetic construct
  REGION 1..15: note = Synthetic construct
WYQQKSNTSPKLWIY

SEQ ID NO: 72 - protein, 32 aa, synthetic construct
  REGION 1..32: note = Synthetic construct
GVPGRFSGSGSGNSYSLTISSMEAEDFATYYC

SEQ ID NO: 73 - protein, 10 aa, synthetic construct
  REGION 1..10: note = Synthetic construct
FGSGTKLELK

SEQ ID NO: 74 - protein, 25 aa, synthetic construct
  REGION 1..25: note = Synthetic construct
EVQLQQSGPELVKPGASVKMSCKAS

SEQ ID NO: 75 - protein, 14 aa, synthetic construct
  REGION 1..14: note = Synthetic construct
WMKQKPGQGLEWIG

SEQ ID NO: 76 - protein, 30 aa, synthetic construct
  REGION 1..30: note = Synthetic construct
KATLTSDKSSNTAYMELSSLTSEDSAVYYC

SEQ ID NO: 77 - protein, 11 aa, synthetic construct
  REGION 1..11: note = Synthetic construct
WGQGTTLTVSS

SEQ ID NO: 78 - protein, 23 aa, synthetic construct
  REGION 1..23: note = Synthetic construct
QIVLTQSPAIMSASPGEKVTMTC

SEQ ID NO: 79 - protein, 15 aa, synthetic construct
  REGION 1..15: note = Synthetic construct
WYQQKSGTSPKKWIY

SEQ ID NO: 80 - protein, 32 aa, synthetic construct
  REGION 1..32: note = Synthetic construct
GVPARFSGSGSGTSYSLTIGSMEAEDAATYYC

SEQ ID NO: 81 - protein, 10 aa, synthetic construct
  REGION 1..10: note = Synthetic construct
FGGGTKLEIK

SEQ ID NO: 82 - protein, 120 aa, synthetic construct
  REGION 1..120: note = Synthetic construct
EVQLVESGPGLVKPSETLSLTCTVSGFSLTRFGVHWVRQPPGKGLEWLGVIWRGGSTDYNAAFMSRLTISKDNSKNQVSLKLSSVTAADTAVYYCSNHYYGSSDYALDNWGQGTLVTVSS

SEQ ID NO: 83 - protein, 107 aa, synthetic construct
  REGION 1..107: note = Synthetic construct
DIQMTQSPSSLSASVGDRVTITCKASQDVSNIVVWFQQKPGKSPKLLIYSASYRYTGVPSRFSGSGSGTDFTLTISSLQPEDFATYYCQQHYSSPYTFGQGTKVEIK

SEQ ID NO: 84 - protein, 120 aa, synthetic construct; identical to SEQ ID NO: 82
  REGION 1..120: note = Synthetic construct

SEQ ID NO: 85 - protein, 107 aa, synthetic construct
  REGION 1..107: note = Synthetic construct
DIQMTQSPSSLSASVGDRVTITCKASQDVRNLVVWFQQKPGKAPKLLIYSGSYRYSGVPSRFSGSGSGTDFTLTISSLQPEDFATYYCQQQYSPPYTFGQGTKVEIK

SEQ ID NO: 86 - protein, 120 aa, synthetic construct; identical to SEQ ID NO: 82
  REGION 1..120: note = Synthetic construct

SEQ ID NO: 87 - protein, 107 aa, synthetic construct
  REGION 1..107: note = Synthetic construct
DIQMTQSPSSLSASVGDRVTITCKASQDVRNLVVWFQQKPGKAPKLLIYSGYNRYSGVPSRFSGSGSGTDFTLTISSLQPEDFATYYCQQQFQPPYTFGQGTKVEIK

SEQ ID NO: 88 - protein, 120 aa, synthetic construct; identical to SEQ ID NO: 82
  REGION 1..120: note = Synthetic construct

SEQ ID NO: 89 - protein, 107 aa, synthetic construct
  REGION 1..107: note = Synthetic construct
DIQMTQSPSSLSASVGDRVTITCKASQDVRNIVVWFQQKPGKAPKLLIYSGSYRYSGVPSRFSGSGSGTDFTLTISSLQPEDFATYYCQQQYSPPYTFGQGTKVEIK

SEQ ID NO: 90 - protein, 120 aa, synthetic construct; identical to SEQ ID NO: 82
  REGION 1..120: note = Synthetic construct

SEQ ID NO: 91 - protein, 107 aa, synthetic construct
  REGION 1..107: note = Synthetic construct
DIQMTQSPSSLSASVGDRVTITCKASQDVRNLVVWFQQKPGKAPKLLIYSGSYRYSGVPSRFSGSGSGTDFTLTISSLQPEDFATYYCQQHYSPPYTFGQGTKVEIK

SEQ ID NO: 92 - protein, 120 aa, synthetic construct; identical to SEQ ID NO: 82
  REGION 1..120: note = Synthetic construct

SEQ ID NO: 93 - protein, 107 aa, synthetic construct
  REGION 1..107: note = Synthetic construct
DIQMTQSPSSLSASVGDRVTITCKASQDVSNIVVWFQQKPGKSPKLLIYSGYYRYTGVPSRFSGSGSGTDFTLTISSLQPEDFATYYCQQQFQPPYTFGQGTKVEIK

SEQ ID NO: 94 - protein, 120 aa, synthetic construct; identical to SEQ ID NO: 82
  REGION 1..120: note = Synthetic construct

SEQ ID NO: 95 - protein, 107 aa, synthetic construct
  REGION 1..107: note = Synthetic construct
DIQMTQSPSSLSASVGDRVTITCKASQDVSNIVVWFQQKPGKAPKLLIYSGYYRYSGVPSRFSGSGSGTDFTLTISSLQPEDFATYYCQQQYQPPYTFGQGTKVEIK

SEQ ID NO: 96 - protein, 120 aa, synthetic construct
  REGION 1..120: note = Synthetic construct
EVQLVESGPGLVKPSETLSLTCTVSGFSTTRFGVHWVRQPPGKGLEWLGVIWRGGSTDYNAAFMSRLTISKDNSKNQVSLKLSSVTAADTAVYYCSNHYYGSSDYALDNWGQGTLVTVSS

SEQ ID NO: 97 - protein, 107 aa, synthetic construct
  REGION 1..107: note = Synthetic construct
DIQMTQSPSSLSASVGDRVTITCKASQDVRNLVVWFQQKPGKAPKLLIYSGYYRYTGVPSRFSGSGSGTDFTLTISSLQPEDFATYYCQQHYQPPYTFGQGTKVEIK

SEQ ID NO: 98 - protein, 120 aa, synthetic construct
  REGION 1..120: note = Synthetic construct
EVQLVESGPGLVKPSETLSLTCTVSGFSLTRFGVHWVRQPPGKGLEWIGVIWRGGSTDYNAAFMSRLTISKDNSKNQVSLKLSSVTAADTAVYYCSNHYYGSSDYALDNWGQGTLVTVSS

SEQ ID NO: 99 - protein, 107 aa, synthetic construct; identical to SEQ ID NO: 97
  REGION 1..107: note = Synthetic construct

SEQ ID NO: 100 - protein, 120 aa, synthetic construct; identical to SEQ ID NO: 82
  REGION 1..120: note = Synthetic construct

SEQ ID NO: 101 - protein, 107 aa, synthetic construct; identical to SEQ ID NO: 97
  REGION 1..107: note = Synthetic construct

SEQ ID NO: 102 - protein, 120 aa, synthetic construct
  REGION 1..120: note = Synthetic construct
EVQLVESGPGLVKPSETLSLTCTVSGFSLTRFGVHWVRQPPGKGLEWLGVIWRGGSTDYNAAFVSRLTISKDNSKNQVSLKLSSVTAADTAVYYCSNHYYGSSDYALDNWGQGTLVTVSS

SEQ ID NO: 103 - protein, 107 aa, synthetic construct; identical to SEQ ID NO: 83
  REGION 1..107: note = Synthetic construct

SEQ ID NO: 104 - protein, 120 aa, synthetic construct; identical to SEQ ID NO: 102
  REGION 1..120: note = Synthetic construct

SEQ ID NO: 105 - protein, 107 aa, synthetic construct; identical to SEQ ID NO: 91
  REGION 1..107: note = Synthetic construct

SEQ ID NO: 106 - protein, 120 aa, synthetic construct
  REGION 1..120: note = Synthetic construct
EVQLVESGPGLVKPSETLSLTCTVSGFSTTRFGVHWVRQPPGKGLEWLGVIWRGGSTDYNAAFVSRLTISKDNSKNQVSLKLSSVTAADTAVYYCSNHYYGSPDYALDNWGQGTLVTVSS

SEQ ID NO: 107 - protein, 107 aa, synthetic construct
  REGION 1..107: note = Synthetic construct
DIQMTQSPSSLSASVGDRVTITCKASQDVSNLVVWFQQKPGKAPKLLIYSGSYRYSGVPSRFSGSGSGTDFTLTISSLQPEDFATYYCQQHYSPPYTFGQGTKVEIK

SEQ ID NO: 108 - protein, 119 aa, synthetic construct
  REGION 1..119: note = Synthetic construct
EVQLVESGGGLVQPGGSLRLSCAVSGIDLSSYAMGWVRQAPGKGLEWIGTIGTGGTPYYASWAKGRFTISKDSSKNTVYLQMNSLRAEDTAVYFCARDMYTGSIYYDMWGQGTLVTVSS

SEQ ID NO: 109 - protein, 111 aa, synthetic construct
  REGION 1..111: note = Synthetic construct
DAQLTQSPSSLSASVGDRVTITCQSSQSVFNNAQLSWYQQKPGKPPKLLIYDTSNLASGVPSRFSGSGSGTDFTLTISSLQPEDFATYYCLGAYTDDADNAFGQGTKVEIK

SEQ ID NO: 110 - protein, 118 aa, synthetic construct
  REGION 1..118: note = Synthetic construct
QVQLQQSGPELVRPGVSVKISCKGSGYTFTHYAMHWVKQSHTKSLEWIGMISSSSGNTNFNQKFMDKATMTVDKSSTTAYLELARLTFGDSAIYYCARWSYYALFDYWGQGTTVTVSS

SEQ ID NO: 111 - protein, 106 aa, synthetic construct
  REGION 1..106: note = Synthetic construct
ENVLTQSPAIMSASPGEKVTMTCSADSSVDYIHWYQQKSNTSPKLWIYDTSKLASGVPGRFSGSGSGNSYSLTISSMEAEDFATYYCFQGSGYPLTFGSGTKLELK

SEQ ID NO: 112 - protein, 118 aa, synthetic construct
  REGION 1..118: note = Synthetic construct
EVQLQQSGPELVKPGASVKMSCKASGYTFTNYVIHWMKQKPGQGLEWIGYISPYNDYTKYNEKFEGKATLTSDKSSNTAYMELSSLTSEDSAVYYCARRDYYGSSDYWGQGTTLTVSS

SEQ ID NO: 113 - protein, 106 aa, synthetic construct
  REGION 1..106: note = Synthetic construct
QIVLTQSPAIMSASPGEKVTMTCSASSSVDYMHWYQQKSGTSPKKWIYDTSKLASGVPARFSGSGSGTSYSLTIGSMEAEDAATYYCQQWSSNPPTFGGGTKLEIK

SEQ ID NO: 114 - protein, 977 aa, Homo sapiens
MLLWVILLVLAPVSGQFARTPRPIIFLQPPWTTVFQGERVTLTCKGFRFYSPQKTKWYHRYLGKEILRETPDNILEVQESGEYRCQAQGSPLSSPVHLDFSSASLILQAPLSVFEGDSVVLRCRAKAEVTLNNTIYKNDNVLAFLNKRTDFHIPHACLKDNGAYRCTGYKESCCPVSSNTVKIQVQEPFTRPVLRASSFQPISGNPVTLTCETQLSLERSDVPLRFRFFRDDQTLGLGWSLSPNFQITAMWSKDSGFYWCKAATMPYSVISDSPRSWIQVQIPASHPVLTLSPEKALNFEGTKVTLHCETQEDSLRTLYRFYHEGVPLRHKSVRCERGASISFSLTTENSGNYYCTADNGLGAKPSKAVSLSVTVPVSHPVLNLSSPEDLIFEGAKVTLHCEAQRGSLPILYQFHHEGAALERRSANSAGGVAISFSLTAEHSGNYYCTADNGFGPQRSKAVSLSVTVPVSHPVLTLSSAEALTFEGATVTLHCEVQRGSPQILYQFYHEDMPLWSSSTPSVGRVSFSFSLTEGHSGNYYCTADNGFGPQRSEVVSLFVTVPVSRPILTLRVPRAQAVVGDLLELHCEAPRGSPPILYWFYHEDVTLGSSSAPSGGEASFNLSLTAEHSGNYSCEANNGLVAQHSDTISLSVIVPVSRPILTFRAPRAQAVVGDLLELHCEALRGSSPILYWFYHEDVTLGKISAPSGGGASFNLSLTTEHSGIYSCEADNGLEAQRSEMVTLKVAVPVSRPVLTLRAPGTHAAVGDLLELHCEALRGSPLILYRFFHEDVTLGNRSSPSGGASLNLSLTAEHSGNYSCEADNGLGAQRSETVTLYITGLTANRSGPFATGVAGGLLSIAGLAAGALLLYCWLSRKAGRKPASDPARSPSDSDSQEPTYHNVPAWEELQPVYTNANPRGENVVYSEVRIIQEKKKHAVASDPRHLRNKGSPIIYSEVKVASTPVSGSLFLASSAPHR

SEQ ID NO: 115 - protein, 5 aa, synthetic construct
  REGION 1..5: note = Synthetic construct
SYYIH

SEQ ID NO: 116 - protein, 17 aa, synthetic construct
  REGION 1..17: note = Synthetic construct
WIYPENDNTKYNEKFKD

SEQ ID NO: 117 - protein, 10 aa, synthetic construct
  REGION 1..10: note = Synthetic construct
  SITE 6: note = MISC_FEATURE - X is Y or A
DGYSRXYFDY

SEQ ID NO: 118 - protein, 17 aa, synthetic construct
  REGION 1..17: note = Synthetic construct
KSSQSLLNSRTRKNYLA

SEQ ID NO: 119 - protein, 7 aa, synthetic construct
  REGION 1..7: note = Synthetic construct
WTSTRKS

SEQ ID NO: 120 - protein, 8 aa, synthetic construct
  REGION 1..8: note = Synthetic construct
  SITE 1: note = MISC_FEATURE - X is K or T
XQSFILRT

SEQ ID NO: 121 - protein, 10 aa, synthetic construct
  REGION 1..10: note = Synthetic construct
DGYSRYYFDY

SEQ ID NO: 122 - protein, 10 aa, synthetic construct
  REGION 1..10: note = Synthetic construct
DGYSRAYFDY

SEQ ID NO: 123 - protein, 8 aa, synthetic construct
  REGION 1..8: note = Synthetic construct
KQSFILRT

SEQ ID NO: 124 - protein, 8 aa, synthetic construct
  REGION 1..8: note = Synthetic construct
TQSFILRT

SEQ ID NO: 125 - protein, 30 aa, synthetic construct
  REGION 1..30: note = Synthetic construct
EVQLVQSGAEVKKPGASVKVSCKASGFTFT

SEQ ID NO: 126 - protein, 14 aa, synthetic construct
  REGION 1..14: note = Synthetic construct
WVRQAPGQGLEWIG

SEQ ID NO: 127 - protein, 32 aa, synthetic construct
  REGION 1..32: note = Synthetic construct
RVTITADTSTSTAYLELSSLRSEDTAVYYCAR

SEQ ID NO: 128 - protein, 11 aa, synthetic construct
  REGION 1..11: note = Synthetic construct
WGQGTLVTVSS

SEQ ID NO: 129 - protein, 23 aa, synthetic construct
  REGION 1..23: note = Synthetic construct
DIVMTQSPDSLAVSLGERATINC

SEQ ID NO: 130 - protein, 15 aa, synthetic construct
  REGION 1..15: note = Synthetic construct
WYQQKPGQSPKLLIY

SEQ ID NO: 131 - protein, 32 aa, synthetic construct
  REGION 1..32: note = Synthetic construct
GVPDRFSGSGSGTDFTLTISSLQAEDVAVYYC

SEQ ID NO: 132 - protein, 10 aa, synthetic construct
  REGION 1..10: note = Synthetic construct
FGQGTKVEIK

SEQ ID NO: 133 - protein, 119 aa, synthetic construct
  REGION 1..119: note = Synthetic construct
EVQLVQSGAEVKKPGASVKVSCKASGFTFTSYYIHWVRQAPGQGLEWIGWIYPENDNTKYNEKFKDRVTITADTSTSTAYLELSSLRSEDTAVYYCARDGYSRYYFDYWGQGTLVTVSS

SEQ ID NO: 134 - protein, 112 aa, synthetic construct
  REGION 1..112: note = Synthetic construct
DIVMTQSPDSLAVSLGERATINCKSSQSLLNSRTRKNYLAWYQQKPGQSPKLLIYWTSTRKSGVPDRFSGSGSGTDFTLTISSLQAEDVAVYYCKQSFILRTFGQGTKVEIK

SEQ ID NO: 135 - protein, 119 aa, synthetic construct
  REGION 1..119: note = Synthetic construct
EVQLVQSGAEVKKPGASVKVSCKASGFTFTSYYIHWVRQAPGQGLEWIGWIYPENDNTKYNEKFKDRVTITADTSTSTAYLELSSLRSEDTAVYYCARDGYSRAYFDYWGQGTLVTVSS

SEQ ID NO: 136 - protein, 112 aa, synthetic construct; identical to SEQ ID NO: 134
  REGION 1..112: note = Synthetic construct

SEQ ID NO: 137 - protein, 119 aa, synthetic construct; identical to SEQ ID NO: 133
  REGION 1..119: note = Synthetic construct

SEQ ID NO: 138 - protein, 112 aa, synthetic construct
  REGION 1..112: note = Synthetic construct
DIVMTQSPDSLAVSLGERATINCKSSQSLLNSRTRKNYLAWYQQKPGQSPKLLIYWTSTRKSGVPDRFSGSGSGTDFTLTISSLQAEDVAVYYCTQSFILRTFGQGTKVEIK

SEQ ID NO: 139 - protein, 5 aa, synthetic construct
  REGION 1..5: note = Synthetic construct
NYYIH

SEQ ID NO: 140 - protein, 17 aa, synthetic construct
  REGION 1..17: note = Synthetic construct
WIYPGDGNTKYNEKFKG

SEQ ID NO: 141 - protein, 10 aa, synthetic construct
  REGION 1..10: note = Synthetic construct
DSYSNYYFDY

SEQ ID NO: 142 - protein, 17 aa, synthetic construct
  REGION 1..17: note = Synthetic construct
KSSQSLLNSRTRKNYLA

SEQ ID NO: 143 - protein, 7 aa, synthetic construct
  REGION 1..7: note = Synthetic construct
WASTRES

SEQ ID NO: 144 - protein, 8 aa, synthetic construct
  REGION 1..8: note = Synthetic construct
TQSFILRT

SEQ ID NO: 145 - protein, 30 aa, synthetic construct
  REGION 1..30: note = Synthetic construct
EVQLVQSGAEVKKPGASVKVSCKASGYTFT

SEQ ID NO: 146 - protein, 14 aa, synthetic construct
  REGION 1..14: note = Synthetic construct
WVRQAPGQGLEWIG

SEQ ID NO: 147 - protein, 32 aa, synthetic construct
  REGION 1..32: note = Synthetic construct
RATLTADTSTSTAYLELSSLRSEDTAVYYCAR

SEQ ID NO: 148 - protein, 11 aa, synthetic construct
  REGION 1..11: note = Synthetic construct
WGQGTLVTVSS

SEQ ID NO: 149 - protein, 23 aa, synthetic construct
  REGION 1..23: note = Synthetic construct
DIVMTQSPDSLAVSLGERATINC

SEQ ID NO: 150 - protein, 15 aa, synthetic construct
  REGION 1..15: note = Synthetic construct
WYQQKPGQPPKLLIY

SEQ ID NO: 151 - protein, 32 aa, synthetic construct; identical to SEQ ID NO: 131
  REGION 1..32: note = Synthetic construct

SEQ ID NO: 152 - protein, 10 aa, synthetic construct
  REGION 1..10: note = Synthetic construct
FGQGTKVEIK

SEQ ID NO: 153 - protein, 119 aa, synthetic construct
  REGION 1..119: note = Synthetic construct
EVQLVQSGAEVKKPGASVKVSCKASGYTFTNYYIHWVRQAPGQGLEWIGWIYPGDGNTKYNEKFKGRATLTADTSTSTAYLELSSLRSEDTAVYYCARDSYSNYYFDYWGQGTLVTVSS

SEQ ID NO: 154 - protein, 112 aa, synthetic construct
  REGION 1..112: note = Synthetic construct
DIVMTQSPDSLAVSLGERATINCKSSQSLLNSRTRKNYLAWYQQKPGQPPKLLIYWASTRESGVPDRFSGSGSGTDFTLTISSLQAEDVAVYYCTQSFILRTFGQGTKVEIK

SEQ ID NO: 155 - protein, 5 aa, synthetic construct
  REGION 1..5: note = Synthetic construct
GYTMN

SEQ ID NO: 156 - protein, 17 aa, synthetic construct
  REGION 1..17: note = Synthetic construct
  SITE 9: note = MISC_FEATURE - X is S or T
  SITE 12: note = MISC_FEATURE - X is N or A
  SITE 13: note = MISC_FEATURE - X is Q or D
  SITE 14: note = MISC_FEATURE - X is K or S
  SITE 15: note = MISC_FEATURE - X is V or F
  SITE 17: note = MISC_FEATURE - X is G or D
LINPYKGVXTYXXXXKX

SEQ ID NO: 157 - protein, 13 aa, synthetic construct
  REGION 1..13: note = Synthetic construct
SGYYGDSDWYFDV

SEQ ID NO: 158 - protein, 11 aa, synthetic construct
  REGION 1..11: note = Synthetic construct
RASQDIRNYLN

SEQ ID NO: 159 - protein, 7 aa, synthetic construct
  REGION 1..7: note = Synthetic construct
YTSRLES

SEQ ID NO: 160 - protein, 9 aa, synthetic construct
  REGION 1..9: note = Synthetic construct
QQGNTLPWT

SEQ ID NO: 161 - protein, 17 aa, synthetic construct
  REGION 1..17: note = Synthetic construct
LINPYKGVTTYADSVKG

SEQ ID NO: 162 - protein, 17 aa, synthetic construct
  REGION 1..17: note = Synthetic construct
LINPYKGVSTYNQKFKD

SEQ ID NO: 163 - protein, 17 aa, synthetic construct
  REGION 1..17: note = Synthetic construct
LINPYKGVSTYADSVKG

SEQ ID NO: 164 - protein, 30 aa, synthetic construct
  REGION 1..30: note = Synthetic construct
EVQLVESGGGLVQPGGSLRLSCAASGYSFT

SEQ ID NO: 165 - protein, 14 aa, synthetic construct
  REGION 1..14: note = Synthetic construct
WVRQAPGKDLEWVA

SEQ ID NO: 166 - protein, 32 aa, synthetic construct
  REGION 1..32: note = Synthetic construct
RFTISVDKSKNTAYLQMNSLRAEDTAVYYCAR

SEQ ID NO: 167 - protein, 11 aa, synthetic construct
  REGION 1..11: note = Synthetic construct
WGQGTLVTVSS

SEQ ID NO: 168 - protein, 23 aa, synthetic construct
  REGION 1..23: note = Synthetic construct
DIQMTQSPSSLSASVGDRVTITC

SEQ ID NO: 169 - protein, 15 aa, synthetic construct
  REGION 1..15: note = Synthetic construct
WYQQKPGKAPKLLIY

SEQ ID NO: 170 - protein, 32 aa, synthetic construct
  REGION 1..32: note = Synthetic construct
GVPSRFSGSGSGTDYTLTISSLQPEDFATYYC

SEQ ID NO: 171 - protein, 10 aa, synthetic construct
  REGION 1..10: note = Synthetic construct
FGQGTKLELK

SEQ ID NO: 172 - protein, 122 aa, synthetic construct
  REGION 1..122: note = Synthetic construct
EVQLVESGGGLVQPGGSLRLSCAASGYSFTGYTMNWVRQAPGKDLEWVALINPYKGVSTYNQKFKDRFTISVDKSKNTAYLQMNSLRAEDTAVYYCARSGYYGDSDWYFDVWGQGTLVTVSS

SEQ ID NO: 173 - protein, 107 aa, synthetic construct
  REGION 1..107: note = Synthetic construct
DIQMTQSPSSLSASVGDRVTITCRASQDIRNYLNWYQQKPGKAPKLLIYYTSRLESGVPSRFSGSGSGTDYTLTISSLQPEDFATYYCQQGNTLPWTFGQGTKLELK

SEQ ID NO: 174 - protein, 28 aa, synthetic construct
  REGION 1..28: note = Synthetic construct
QDGNEEMGGITQTPYKVSISGTTVILTC

SEQ ID NO: 175 - protein, 16 aa, synthetic construct
  REGION 1..16: note = Synthetic construct
VIWRGGSTDYNPAFMS

SEQ ID NO: 176 - protein, 16 aa, synthetic construct
  REGION 1..16: note = Synthetic construct
VIWRGGSTDYNAAFGS

SEQ ID NO: 177 - protein, 16 aa, synthetic construct
  REGION 1..16: note = Synthetic construct
VIWRGGSTDYNAAFMD

SEQ ID NO: 178 - protein, 16 aa, synthetic construct
  REGION 1..16: note = Synthetic construct
VIWRGGSTDYNAAFMP

SEQ ID NO: 179 - protein, 30 aa, synthetic construct
  REGION 1..30: note = Synthetic construct
SVQLVESGPGLVKPSETLSLTCTVSGFSLT

SEQ ID NO: 180 - protein, 30 aa, synthetic construct
  REGION 1..30: note = Synthetic construct
FVQLVESGPGLVKPSETLSLTCTVSGFSLT

SEQ ID NO: 181 - protein, 30 aa, synthetic construct
  REGION 1..30: note = Synthetic construct
EVQLVESGPGLVKPSETLSLTCTVSGFPLT

SEQ ID NO: 182 - protein, 14 aa, synthetic construct
  REGION 1..14: note = Synthetic construct
WYRQPPGKGLEWLG

SEQ ID NO: 183 - protein, 32 aa, synthetic construct
  REGION 1..32: note = Synthetic construct
RLTISKDNSKNQVSLMLSSVTAADTAVYYCSN

SEQ ID NO: 184 - protein, 32 aa, synthetic construct
  REGION 1..32: note = Synthetic construct
RLTISKDNSKNQVSLKLSDVTAADTAVYYCSN

SEQ ID NO: 185 - protein, 120 aa, synthetic construct
  REGION 1..120: note = Synthetic construct
SVQLVESGPGLVKPSETLSLTCTVSGFSLTRFGVHWVRQPPGKGLEWLGVIWRGGSTDYNAAFMSRLTISKDNSKNQVSLKLSSVTAADTAVYYCSNHYYGSSDYALDNWGQGTLVTVSS

SEQ ID NO: 186 - protein, 107 aa, synthetic construct; identical to SEQ ID NO: 83
  REGION 1..107: note = Synthetic construct

SEQ ID NO: 187 - protein, 120 aa, synthetic construct
  REGION 1..120: note = Synthetic construct
FVQLVESGPGLVKPSETLSLTCTVSGFSLTRFGVHWVRQPPGKGLEWLGVIWRGGSTDYNAAFMSRLTISKDNSKNQVSLKLSSVTAADTAVYYCSNHYYGSSDYALDNWGQGTLVTVSS

SEQ ID NO: 188 - protein, 107 aa, synthetic construct; identical to SEQ ID NO: 83
  REGION 1..107: note = Synthetic construct

SEQ ID NO: 189 - protein, 120 aa, synthetic construct
  REGION 1..120: note = Synthetic construct
EVQLVESGPGLVKPSETLSLTCTVSGFPLTRFGVHWVRQPPGKGLEWLGVIWRGGSTDYNAAFMSRLTISKDNSKNQVSLKLSSVTAADTAVYYCSNHYYGSSDYALDNWGQGTLVTVSS

SEQ ID NO: 190 - protein, 107 aa, synthetic construct; identical to SEQ ID NO: 83
  REGION 1..107: note = Synthetic construct

SEQ ID NO: 191 - protein, 120 aa, synthetic construct; identical to SEQ ID NO: 96
  REGION 1..120: note = Synthetic construct

SEQ ID NO: 192 - protein, 107 aa, synthetic construct; identical to SEQ ID NO: 83
  REGION 1..107: note = Synthetic construct

SEQ ID NO: 193 - protein, 120 aa, synthetic construct
  REGION 1..120: note = Synthetic construct
EVQLVESGPGLVKPSETLSLTCTVSGFSLTRFGVHWYRQPPGKGLEWLGVIWRGGSTDYNAAFMSRLTISKDNSKNQVSLKLSSVTAADTAVYYCSNHYYGSSDYALDNWGQGTLVTVSS

SEQ ID NO: 194 - protein, 107 aa, synthetic construct; identical to SEQ ID NO: 83
  REGION 1..107: note = Synthetic construct

SEQ ID NO: 195 - protein, 120 aa, synthetic construct
  REGION 1..120: note = Synthetic construct
EVQLVESGPGLVKPSETLSLTCTVSGFSLTRFGVHWVRQPPGKGLEWLGVIWRGGSTDYNPAFMSRLTISKDNSKNQVSLKLSSVTAADTAVYYCSNHYYGSSDYALDNWGQGTLVTVSS

SEQ ID NO: 196 - protein, 107 aa, synthetic construct; identical to SEQ ID NO: 83
  REGION 1..107: note = Synthetic construct

SEQ ID NO: 197 - protein, 120 aa, synthetic construct
  REGION 1..120: note = Synthetic construct
EVQLVESGPGLVKPSETLSLTCTVSGFSLTRFGVHWVRQPPGKGLEWLGVIWRGGSTDYNAAFGSRLTISKDNSKNQVSLKLSSVTAADTAVYYCSNHYYGSSDYALDNWGQGTLVTVSS

SEQ ID NO: 198 - protein, 107 aa, synthetic construct; identical to SEQ ID NO: 83
  REGION 1..107: note = Synthetic construct

SEQ ID NO: 199 - protein, 120 aa, synthetic construct
  REGION 1..120: note = Synthetic construct
EVQLVESGPGLVKPSETLSLTCTVSGFSLTRFGVHWVRQPPGKGLEWLGVIWRGGSTDYNAAFMDRLTISKDNSKNQVSLKLSSVTAADTAVYYCSNHYYGSSDYALDNWGQGTLVTVSS

SEQ ID NO: 200 - protein, 107 aa, synthetic construct; identical to SEQ ID NO: 83
  REGION 1..107: note = Synthetic construct

SEQ ID NO: 201 - protein, 120 aa, synthetic construct
  REGION 1..120: note = Synthetic construct
EVQLVESGPGLVKPSETLSLTCTVSGFSLTRFGVHWVRQPPGKGLEWLGVIWRGGSTDYNAAFMPRLTISKDNSKNQVSLKLSSVTAADTAVYYCSNHYYGSSDYALDNWGQGTLVTVSS

SEQ ID NO: 202 - protein, 107 aa, synthetic construct; identical to SEQ ID NO: 83
  REGION 1..107: note = Synthetic construct

SEQ ID NO: 203 - protein, 120 aa, synthetic construct
  REGION 1..120: note = Synthetic construct
EVQLVESGPGLVKPSETLSLTCTVSGFSLTRFGVHWVRQPPGKGLEWLGVIWRGGSTDYNAAFMSRLTISKDNSKNQVSLMLSSVTAADTAVYYCSNHYYGSSDYALDNWGQGTLVTVSS

SEQ ID NO: 204 - protein, 107 aa, synthetic construct; identical to SEQ ID NO: 83
  REGION 1..107: note = Synthetic construct

SEQ ID NO: 205 - protein, 120 aa, synthetic construct
  REGION 1..120: note = Synthetic construct
EVQLVESGPGLVKPSETLSLTCTVSGFSLTRFGVHWVRQPPGKGLEWLGVIWRGGSTDYNAAFMSRLTISKDNSKNQVSLKLSDVTAADTAVYYCSNHYYGSSDYALDNWGQGTLVTVSS

SEQ ID NO: 206 - protein, 107 aa, synthetic construct; identical to SEQ ID NO: 83
  REGION 1..107: note = Synthetic construct

SEQ ID NO: 207 - protein, 120 aa, synthetic construct
  REGION 1..120: note = Synthetic construct
EVQLVESGPGLVKPSETLSLTCTVSGFSLTRFGVHWVRQPPGKGLEWLGVIWRGGSTDYNAAFMSRLTISKDNSKNQVSLKLSSVTAADTAVYYCSNHYYGSPDYALDNWGQGTLVTVSS

SEQ ID NO: 208 - protein, 107 aa, synthetic construct; identical to SEQ ID NO: 83
  REGION 1..107: note = Synthetic construct

SEQ ID NO: 209 - protein, 120 aa, synthetic construct; identical to SEQ ID NO: 102
  REGION 1..120: note = Synthetic construct

SEQ ID NO: 210 - protein, 107 aa, synthetic construct
  REGION 1..107: note = Synthetic construct
DIQMTQSPSSLSASVGDRVTITCKASQDVSNLVVWFQQKPGKSPKLLIYSGSYRYSGVPSRFSGSGSGTDFTLTISSLQPEDFATYYCQQHYSPPYTFGQGTKVEIK

SEQ ID NO: 211 - protein, 120 aa, synthetic construct
  REGION 1..120: note = Synthetic construct
EVQLVESGPGLVKPSETLSLTCTVSGFSTTRFGVHWVRQPPGKGLEWLGVIWRGGSTDYNAAFVSRLTISKDNSKNQVSLKLSSVTAADTAVYYCSNHYYGSSDYALDNWGQGTLVTVSS

SEQ ID NO: 212 - protein, 107 aa, synthetic construct; identical to SEQ ID NO: 210
  REGION 1..107: note = Synthetic construct

SEQ ID NO: 213 - protein, 120 aa, synthetic construct
  REGION 1..120: note = Synthetic construct
EVQLVESGPGLVKPSETLSLTCTVSGFSLTRFGVHWVRQPPGKGLEWLGVIWRGGSTDYNAAFVSRLTISKDNSKNQVSLKLSSVTAADTAVYYCSNHYYGSPDYALDNWGQGTLVTVSS

SEQ ID NO: 214 - protein, 107 aa, synthetic construct; identical to SEQ ID NO: 210
  REGION 1..107: note = Synthetic construct

SEQ ID NO: 215 - protein, 975 aa, Macaca fascicularis
MLLWVILLVLAPVSGQFVRTYKSHFLQPPWTTVFRGERVNLTCKGFGFYSSQKTKWYYRHLGKEISRETQKNTLEVQESGEYRCQAQGSPLSSPVSLDFSSASLILQAPLSVFEGDSVVLRCRAKAEVTLKTTIYKNENVLAFLNKSTDFHISHASLKDNGAYRCTGYKETCCLVSSNTVKIQVQESFTRPVLRVSSFQPISGSPVTLTCETQLSLERSDVPLQFCFFRNDQMLGSGCSLSPKFRITAMWSKDSGSYWCKAATMCYDTTSNSLRSWIQVLIPASHPVLTLSPEKALNFEGTKVKLHCETQEDSLRTLYKFYHDGVPLRYKSVRCEKGASISFSLTTEHSGNYYCTADNGHGAKPSEAVSLSVTVPVSRPVLTLSSAEDLISEGAKLTLHCEAQRGSLPIVYQFHHENASLGNRSAHSAGGVAISFSLTADHSGNYYCTANNGFGPQRSEAVSLSITVPVSRPVLTLSSAEALTFEGATVTLYCEVQRGSPRILYQFYHEDVPLGSNSTPSVGKVSFSFSLTAAHSGNYYCTADNGFGPQRSEAVSLFVTVPVSRPILTLRVPRAQAVVGDLLELRCEALRGSPPIMYWFYHEDVTLGSSSVPSGGEASFNLSLTAEHSGNYSCEANNGLVAQHSDTISLSVIVPVSRPILTFRAPRAQAVVGDLLELHCEALRGSSPILYWFYHEDVTLGKISAPSGGGAYFNLSLTTEHSGIYSCEADNGLEAQRSEMVTLKVAVPVSRPVLTLRAPRAQVAVGDLLELHCEALRGSPLILYQFYHEDVTLGNSSALSGGAFFNLSLTAEHGNYSCEADNGLGAQRSETVTLYLTGLTENRSGPVATGVTGGLLSLAGLAAVALLLYCWLSRKAGREPASDPCRSPSDLDSQEPTYHNVPAWEELQPVYSNVNPRGENVVYSEVRIIREKKKHAVASNPRHLRNKGSCIIYSEVKVASTPASRCLFLASSAPHR